European Patent Specification EP 3 643 706 B1, published November 15, 2023. Title: Modified nucleic acid monomer compound and oligonucleic acid analog. Applicant: EISAI R & D MANAGEMENT Co., Ltd. The sequence listing filed with the application follows.

SEQUENCE LISTING (34 sequences)

SEQ ID NO: 1 - RNA, 19 nt, Artificial Sequence
  #1 sense
  misc_feature (1)..(1): n stands for a nucleotide unit derived from compound 22'
ncuaugggcugaauacaaa

SEQ ID NO: 2 - RNA, 19 nt, Artificial Sequence
  #1 antisense
uuuguauucagcccauagc

SEQ ID NO: 3 - RNA, 19 nt, Artificial Sequence
  #2 sense
  misc_feature (19)..(19): n stands for a nucleotide unit derived from compound 27'(b)
gcuaugggcugaauacaan

SEQ ID NO: 4 - RNA, 19 nt, Artificial Sequence
  #2 antisense
uuuguauucagcccauagc

SEQ ID NO: 5 - RNA, 19 nt, Artificial Sequence
  #3 sense
  misc_feature (1)..(1): n stands for a nucleotide unit derived from compound 22'
  misc_feature (19)..(19): n stands for a nucleotide unit derived from compound 27'(b)
ncuaugggcugaauacaan

SEQ ID NO: 6 - RNA, 19 nt, Artificial Sequence
  #3 antisense
uuuguauucagcccauagc

SEQ ID NO: 7 - RNA, 19 nt, Artificial Sequence
  #4 sense
  misc_feature (1)..(1): n stands for a nucleotide unit derived from compound 22'
  misc_feature (2)..(2): n stands for a nucleotide  unit derived from compound 20'
nnuaugggcugaauacaaa

SEQ ID NO: 8 - RNA, 19 nt, Artificial Sequence
  #4 antisense
uuuguauucagcccauagc

SEQ ID NO: 9 - RNA, 19 nt, Artificial Sequence
  #5 sense
  misc_feature (18)..(18): n stands for a nucleotide unit derived from comound 27'(a)
  misc_feature (19)..(19): n stands for a nucleotide unit derived from compound 27'(b)
gcuaugggcugaauacann

SEQ ID NO: 10 - RNA, 19 nt, Artificial Sequence
  #5 antisense
uuuguauucagcccauagc

SEQ ID NO: 11 - RNA, 19 nt, Artificial Sequence
  #6 sense
  misc_feature (1)..(1): n stands for a nucleotide unit derived from compound 20'
  misc_feature (19)..(19): n stands for a nucleotide unit derived from compound 8'(b)
ngaucauacaaaagaucan

SEQ ID NO: 12 - RNA, 19 nt, Artificial Sequence
  #6 antisense
augaucuuuuguaugaucg

SEQ ID NO: 13 - RNA, 19 nt, Artificial Sequence
  #7 sense
  misc_feature (1)..(1): n stands for a nucleotide unit derived from compound 20'
  misc_feature (2)..(2): n stands for a nucleotide unit derived from compound 22'
nnaucauacaaaagaucau

SEQ ID NO: 14 - RNA, 19 nt, Artificial Sequence
  #7 antisense
augaucuuuuguaugaucg

SEQ ID NO: 15 - RNA, 19 nt, Artificial Sequence
  #8 sense
  misc_feature (1)..(1): n stands for a nucleotide unit derived from compound 20'
  misc_feature (2)..(2): n stands for a nucleotide unit derived from compound 22'
  misc_feature (18)..(18): n stands for a nucleotide unit derived from compound 27'(a)
  misc_feature (19)..(19): n stands for a nucleotide unit derived from compound 8'(b)
nnaucauacaaaagaucnn

SEQ ID NO: 16 - RNA, 19 nt, Artificial Sequence
  #8 antisense
augaucuuuuguaugaucg

SEQ ID NO: 17 - DNA, 21 bp, Artificial Sequence
  #9 sense
  misc_difference (1)..(19): RNA
  misc_difference (20)..(21): DNA
cgaucauacaaaagaucautt

SEQ ID NO: 18 - DNA, 21 bp, Artificial Sequence
  #9 antisense
  misc_difference (1)..(19): RNA
  misc_feature (7)..(7): n stands for a nucleotide unit derived from compound 8'(a)
  misc_difference (20)..(21): DNA
augaucnuuuguaugaucgtt

SEQ ID NO: 19 - RNA, 19 nt, Artificial Sequence
  #10 sense
  misc_feature (4)..(4): n stands for 2'- fluorouridine
  misc_feature (5)..(5): n stands for 2'- fluorocytidine
  misc_feature (7)..(7): n stands for 2'- fluorouridine
  misc_feature (8)..(8): n stands for 2'- fluorocytidine
  misc_feature (9)..(9): n stands for 2'- fluorouridine
  misc_feature (10)..(10): n stands for 2'- fluorocytidine
  misc_feature (14)..(14): n stands for 2'- fluorouridine
  misc_feature (15)..(15): n stands for 2'- fluorocytidine
  misc_feature (16)..(16): n stands for 2'- fluorouridine
  misc_feature (17)..(17): n stands for 2'- fluorouridine
  misc_feature (19)..(19): n stands for 2'- fluorocytidine
ggannannnnaagnnnnan

SEQ ID NO: 20 - RNA, 21 nt, Artificial Sequence
  #10 antisense
  misc_feature (2)..(2): n stands for 2'- fluorouridine
  misc_feature (7)..(7): n stands for 2'- fluorocytidine
  misc_feature (8)..(8): n stands for 2'- fluorouridine
  misc_feature (9)..(9): n stands for 2'- fluorouridine
  misc_feature (14)..(14): n stands for 2'- fluorouridine
  misc_feature (17)..(17): n stands for 2'- fluorouridine
  misc_feature (18)..(18): n stands for 2'- fluorocytidine
  misc_feature (19)..(19): n stands for 2'- fluorocytidine
  misc_feature (20)..(20): n stands for a nucleotide unit derived from compound 18'(a)
  misc_feature (21)..(21): n stands for a nucleotide unit derived from compound 18'(b)
gnaagannngagangannnnn

SEQ ID NO: 21 - RNA, 19 nt, Artificial Sequence
  Cont-1 sense
gcuaugggcugaauacaaa

SEQ ID NO: 22 - RNA, 19 nt, Artificial Sequence
  Cont-1 antisense
uuuguauucagcccauagc

SEQ ID NO: 23 - DNA, 21 bp, Artificial Sequence
  Cont-2 sense
  misc_difference (1)..(19): RNA
  misc_difference (20)..(21): DNA
cgaucauacaaaagaucautt

SEQ ID NO: 24 - DNA, 21 bp, Artificial Sequence
  Cont-2 antisense
  misc_difference (1)..(19): RNA
  misc_difference (20)..(21): DNA
augaucuuuuguaugaucgtt

SEQ ID NO: 25 - RNA, 19 nt, Artificial Sequence
  Cont-3 sense
cgaucauacaaaagaucau

SEQ ID NO: 26 - RNA, 19 nt, Artificial Sequence
  Cont-3 antisense
augaucuuuuguaugaucg

SEQ ID NO: 27 - RNA, 21 nt, Artificial Sequence
  Cont-4 sense
  misc_binding (20)..(21): phosphorothioate binding
gcuaugggcugaauacaaauu

SEQ ID NO: 28 - RNA, 21 nt, Artificial Sequence
  Cont-4 antisense
  misc_binding (20)..(21): phosphorothioate binding
uuuguauucagcccauagcuu

SEQ ID NO: 29 - RNA, 19 nt, Artificial Sequence
  Cont-5 sense
  misc_feature (4)..(4): n stands for 2'- fluorouridine
  misc_feature (5)..(5): n stands for 2'- fluorocytidine
  misc_feature (7)..(7): n stands for 2'- fluorouridine
  misc_feature (8)..(8): n stands for 2'- fluorocytidine
  misc_feature (9)..(9): n stands for 2'- fluorouridine
  misc_feature (10)..(10): n stands for 2'- fluorocytidine
  misc_feature (14)..(14): n stands for 2'- fluorouridine
  misc_feature (15)..(15): n stands for 2'- fluorocytidine
  misc_feature (16)..(16): n stands for 2'- fluorouridine
  misc_feature (17)..(17): n stands for 2'- fluorouridine
  misc_feature (19)..(19): n stands for 2'- fluorocytidine
ggannannnnaagnnnnan

SEQ ID NO: 30 - RNA, 21 nt, Artificial Sequence
  Cont-5 antisense
  misc_feature (2)..(2): n stands for 2'- fluorouridine
  misc_feature (7)..(7): n stands for 2'- fluorocytidine
  misc_feature (8)..(8): n stands for 2'- fluorouridine
  misc_feature (9)..(9): n stands for 2'- fluorouridine
  misc_feature (14)..(14): n stands for 2'- fluorouridine
  misc_feature (17)..(17): n stands for 2'- fluorouridine
  misc_feature (18)..(18): n stands for 2'- fluorocytidine
  misc_feature (19)..(19): n stands for 2'- fluorocytidine
  modified_base (20)..(20): um
  modified_base (21)..(21): um
gnaagannngagangannnuu

SEQ ID NO: 31 - DNA, 21 bp, Artificial Sequence
  Cont-6 sense
  misc_difference (1)..(19): RNA
  misc_difference (20)..(21): DNA
cgaucauacaaaagaucautt

SEQ ID NO: 32 - DNA, 21 bp, Artificial Sequence
  Cont-6 antisense
  misc_difference (1)..(19): RNA
  misc_feature (7)..(7): n stands for a nucleotide unit derived from compound 43'
  misc_difference (20)..(21): DNA
augaucnuuuguaugaucgtt

SEQ ID NO: 33 - DNA, 21 bp, Artificial Sequence
  Cont-7 sense
  misc_difference (1)..(19): RNA
  misc_difference (20)..(21): DNA
cgaucauacaaaagaucautt

SEQ ID NO: 34 - DNA, 21 bp, Artificial Sequence
  Cont-7 antisense
  misc_difference (1)..(19): RNA
  misc_feature (7)..(7): n stands for a nucleotide unit derived from compound 44'
  misc_difference (20)..(21): DNA
augaucnuuuguaugaucgtt